European Patent Specification EP 3 697 804 B1, published August 23, 2023. Title: Expression of PCV2 ORF2 in insect cells. Applicant: Intervet Int. BV. The sequence listing filed with the application follows.

SEQUENCE LISTING (2 sequences)

SEQ ID NO: 1 - DNA, 702 bp, Artificial Sequence
  PCV2b ORF2 gene - mutated
  CDS (1)..(699)
atgacctacccccgtcgtcgttaccgtcgtcgtcgtcaccgtccccgtagccatctgggccaaatccttcgtcgtcgtccctggctggttcacccccgtcatcgttaccgttggcgtcgtaagaacggtatcttcaacacccgtctttcacgtaccttcggatacactgttaagcgtaccactgtgaaaactcccagctgggctgttgacatgatgcgtttcaacatcaacgacttccttccccccggaggtggaagcaacccccgttctgtgcccttcgagtactaccgtatccgtaaggttaaagtggaattctggccctgctctcccatcacccaaggcgaccgtggcgttggtagctctgccgtgatccttgacgacaacttcgttcccaaagctaccgccctcacttacgacccctacgtgaactactcaagccgtcacaccatcactcaacccttctcttaccattcacgttacttcacccccaagcccgttctcgactctactatcgactacttccaacccaacaacaaacgtaaccaactgtggcttcgtctccaaaccactggtaacgttgaccacgtgggactgggcaccgctttcgagaactcaatctacgaccaagaatacaacatccgtgttactatgtacgtgcaattccgtgagttcaacctcaaggacccccccctgaacccctaa

SEQ ID NO: 2 - protein, 233 aa, Artificial Sequence
  Synthetic Construct
MTYPRRRYRRRRHRPRSHLGQILRRRPWLVHPRHRYRWRRKNGIFNTRLSRTFGYTVKRTTVKTPSWAVDMMRFNINDFLPPGGGSNPRSVPFEYYRIRKVKVEFWPCSPITQGDRGVGSSAVILDDNFVPKATALTYDPYVNYSSRHTITQPFSYHSRYFTPKPVLDSTIDYFQPNNKRNQLWLRLQTTGNVDHVGLGTAFENSIYDQEYNIRVTMYVQFREFNLKDPPLNP